European Patent Specification EP 3 256 126 B1, published March 27, 2024. Title: Compounds for the treatment of cancer. Applicant: F. Hoffmann-La Roche AG. The sequence listing filed with the application follows.

SEQUENCE LISTING (6 sequences)

SEQ ID NO: 1 - protein, 801 aa, Homo sapiens
MKTSPRRPLILKRRRLPLPVQNAPSETSEEEPKRSPAQQESNQAEASKEVAESNSCKFPAGIKIINHPTMPNTQVVAIPNNANIHSIITALTAKGKESGSSGPNKFILISCGGAPTQPPGLRPQTQTSYDAKRTEVTLETLGPKPAARDVNLPRPPGALCEQKRETCADGEAAGCTINNSLSNIQWLRKMSSDGLGSRSIKQEMEEKENCHLEQRQVKVEEPSRPSASWQNSVSERPPYSYMAMIQFAINSTERKRMTLKDIYTWIEDHFPYFKHIAKPGWKNSIRHNLSLHDMFVRETSANGKVSFWTIHPSANRYLTLDQVFKPLDPGSPQLPEHLESQQKRPNPELRRNMTIKTELPLGARRKMKPLLPRVSSYLVPIQFPVNQSLVLQPSVKVPLPLAASLMSSELARHSKRVRIAPKVFGEQVVFGYMSKFFSGDLRDFGTPITSLFNFIFLCLSVLLAEEGIAPLSSAGPGKEEKLLFGEGFSPLLPVQTIKEEEIQPGEEMPHLARPIKVESPPLEEWPSPAPSFKEESSHSWEDSSQSPTPRPKKSYSGLRSPTRCVSEMLVIQHRERRERSRSRRKQHLLPPCVDEPELLFSEGPSTSRWAAELPFPADSSDPASQLSYSQEVGGPFKTPIKETLPISSTPSKSVLPRTPESWRLTPPAKVGGLDFSPVQTSQGASDPLPDPLGLMDLSTTPLQSAPPLESPQRLLSSEPLDLISVPFGNSSPSDIDVPKPGSPEPQVSGLAANRSLTEGLVLDTMNDSLSKILLDISFPGLDEDPLGPDNINWSQFIPELQ

SEQ ID NO: 2 - protein, 748 aa, Homo sapiens
MKTSPRRPLILKRRRLPLPVQNAPSETSEEEPKRSPAQQESNQAEASKEVAESNSCKFPAGIKIINHPTMPNTQVVAIPNNANIHSIITALTAKGKESGSSGPNKFILISCGGAPTQPPGLRPQTQTSYDAKRTEVTLETLGPKPAARDVNLPRPPGALCEQKRETCDGEAAGCTINNSLSNIQWLRKMSSDGLGSRSIKQEMEEKENCHLEQRQVKVEEPSRPSASWQNSVSERPPYSYMAMIQFAINSTERKRMTLKDIYTWIEDHFPYFKHIAKPGWKNSIRHNLSLHDMFVRETSANGKVSFWTIHPSANRYLTLDQVFKQQQKRPNPELRRNMTIKTELPLGARRKMKPLLPRVSSYLVPIQFPVNQSLVLQPSVKVPLPLAASLMSSELARHSKRVRIAPKVLLAEEGIAPLSSAGPGKEEKLLFGEGFSPLLPVQTIKEEEIQPGEEMPHLARPIKVESPPLEEWPSPAPSFKEESSHSWEDSSQSPTPRPKKSYSGLRSPTRCVSEMLVIQHRERRERSRSRRKQHLLPPCVDEPELLFSEGPSTSRWAAELPFPADSSDPASQLSYSQEVGGPFKTPIKETLPISSTPSKSVLPRTPESWRLTPPAKVGGLDFSPVQTSQGASDPLPDPLGLMDLSTTPLQSAPPLESPQRLLSSEPLDLISVPFGNSSPSDIDVPKPGSPEPQVSGLAANRSLTEGLVLDTMNDSLSKILLDISFPGLDEDPLGPDNINWSQFIPELQ

SEQ ID NO: 3 - protein, 763 aa, Homo sapiens
MKTSPRRPLILKRRRLPLPVQNAPSETSEEEPKRSPAQQESNQAEASKEVAESNSCKFPAGIKIINHPTMPNTQVVAIPNNANIHSIITALTAKGKESGSSGPNKFILISCGGAPTQPPGLRPQTQTSYDAKRTEVTLETLGPKPAARDVNLPRPPGALCEQKRETCADGEAAGCTINNSLSNIQWLRKMSSDGLGSRSIKQEMEEKENCHLEQRQVKVEEPSRPSASWQNSVSERPPYSYMAMIQFAINSTERKRMTLKDIYTWIEDHFPYFKHIAKPGWKNSIRHNLSLHDMFVRETSANGKVSFWTIHPSANRYLTLDQVFKPLDPGSPQLPEHLESQQKRPNPELRRNMTIKTELPLGARRKMKPLLPRVSSYLVPIQFPVNQSLVLQPSVKVPLPLAASLMSSELARHSKRVRIAPKVLLAEEGIAPLSSAGPGKEEKLLFGEGFSPLLPVQTIKEEEIQPGEEMPHLARPIKVESPPLEEWPSPAPSFKEESSHSWEDSSQSPTPRPKKSYSGLRSPTRCVSEMLVIQHRERRERSRSRRKQHLLPPCVDEPELLFSEGPSTSRWAAELPFPADSSDPASQLSYSQEVGGPFKTPIKETLPISSTPSKSVLPRTPESWRLTPPAKVGGLDFSPVQTSQGASDPLPDPLGLMDLSTTPLQSAPPLESPQRLLSSEPLDLISVPFGNSSPSDIDVPKPGSPEPQVSGLAANRSLTEGLVLDTMNDSLSKILLDISFPGLDEDPLGPDNINWSQFIPELQ

SEQ ID NO: 4 - DNA, 3665 bp, Homo sapiens
  CDS (284)..(2689)
tttcaaacagcggaacaaactgaaagctccggtgccagaccccacccccggccccggcccgggaccccctcccctcccgggatcccccggggttcccaccccgcccgcaccgccggggacccggccggtccggcgcgagcccccgtccggggccctggctcggcccccaggttggaggagcccggagcccgccttcggagctacggcctaacggcggcggcgactgcagtctggagggtccacacttgtgattctcaatggagagtgaaaacgcagattcataatgaaaactagcccccgtcggccactgattctcaaaagacggaggctgccccttcctgttcaaaatgccccaagtgaaacatcagaggaggaacctaagagatcccctgcccaacaggagtctaatcaagcagaggcctccaaggaagtggcagagtccaactcttgcaagtttccagctgggatcaagattattaaccaccccaccatgcccaacacgcaagtagtggccatccccaacaatgctaatattcacagcatcatcacagcactgactgccaagggaaaagagagtggcagtagtgggcccaacaaattcatcctcatcagctgtgggggagccccaactcagcctccaggactccggcctcaaacccaaaccagctatgatgccaaaaggacagaagtgaccctggagaccttgggaccaaaacctgcagctagggatgtgaatcttcctagaccacctggagccctttgcgagcagaaacgggagacctgtgcagatggtgaggcagcaggctgcactatcaacaatagcctatccaacatccagtggcttcgaaagatgagttctgatggactgggctcccgcagcatcaagcaagagatggaggaaaaggagaattgtcacctggagcagcgacaggttaaggttgaggagccttcgagaccatcagcgtcctggcagaactctgtgtctgagcggccaccctactcttacatggccatgatacaattcgccatcaacagcactgagaggaagcgcatgactttgaaagacatctatacgtggattgaggaccactttccctactttaagcacattgccaagccaggctggaagaactccatccgccacaacctttccctgcacgacatgtttgtccgggagacgtctgccaatggcaaggtctccttctggaccattcaccccagtgccaaccgctacttgacattggaccaggtgtttaagccactggacccagggtctccacaattgcccgagcacttggaatcacagcagaaacgaccgaatccagagctccgccggaacatgaccatcaaaaccgaactccccctgggcgcacggcggaagatgaagccactgctaccacgggtcagctcatacctggtacctatccagttcccggtgaaccagtcactggtgttgcagccctcggtgaaggtgccattgcccctggcggcttccctcatgagctcagagcttgcccgccatagcaagcgagtccgcattgcccccaaggtttttggggaacaggtggtgtttggttacatgagtaagttctttagtggcgatctgcgagattttggtacacccatcaccagcttgtttaattttatctttctttgtttatcagtgctgctagctgaggaggggatagctcctctttcttctgcaggaccagggaaagaggagaaactcctgtttggagaagggttttctcctttgcttccagttcagactatcaaggaggaagaaatccagcctggggaggaaatgccacacttagcgagacccatcaaagtggagagccctcccttggaagagtggccctccccggccccatctttcaaagaggaatcatctcactcctgggaggattcgtcccaatctcccaccccaagacccaagaagtcctacagtgggcttaggtccccaacccggtgtgtctcggaaatgcttgtgattcaacacagggagaggagggagaggagccggtctcggaggaaacagcatctactgcctccctgtgtggatgagccggagctgctcttctcagaggggcccagtacttcccgctgggccgcagagctcccgttcccagcagactcctctgaccctgcctcccagctcagctactcccaggaagtgggaggaccttttaagacacccattaaggaaacgctgcccatctcctccaccccgagcaaatctgtcctccccagaacccctgaatcctggaggctcacgcccccagccaaagtagggggactggatttcagcccagtacaaacctcccagggtgcctctgaccccttgcctgaccccctggggctgatggatctcagcaccactcccttgcaaagtgctcccccccttgaatcaccgcaaaggctcctcagttcagaacccttagacctcatctccgtcccctttggcaactcttctccctcagatatagacgtccccaagccaggctccccggagccacaggtttctggccttgcagccaatcgttctctgacagaaggcctggtcctggacacaatgaatgacagcctcagcaagatcctgctggacatcagctttcctggcctggacgaggacccactgggccctgacaacatcaactggtcccagtttattcctgagctacagtagagccctgcccttgcccctgtgctcaagctgtccaccatcccgggcactccaaggctcagtgcaccccaagcctctgagtgaggacagcaggcagggactgttctgctcctcatagctccctgctgcctgattatgcaaaagtagcagtcacaccctagccactgctgggaccttgtgttccccaagagtatctgattcctctgctgtccctgccaggagctgaagggtgggaacaacaaaggcaatggtgaaaagagattaggaaccccccagcctgtttccattctctgcccagcagtctcttaccttccctgatctttgcagggtggtccgtgtaaatagtataaattctccaaattatcctctaattataaatgtaagcttatttccttagatcattatccagagactgccagaaggtgggtaggatgacctggggtttcaattgacttctgttccttgcttttagttttgatagaagggaagacctgcagtgcacggtttcttccaggctgaggtacctggatcttgggttcttcactgcagggacccagacaagtggatctgcttgccagagtcctttttgcccctccctgccacctccccgtgtttccaagtcagctttcctgcaagaagaaatcctggttaaaaaagtcttttgtattgggtcaggagttgaatttggggtgggaggatggatgcaactgaagcagagtgtgggtgcccagatgtgcgctattagatgtttctctgataatgtccccaatcataccagggagactggcattgacgagaactcaggtggaggcttgagaaggccgaaagggcccctgacctgcctggcttccttagcttgcccctcagctttgcaaagagccaccctaggccccagctgaccgcatgggtgtgagccagcttgagaacactaactactcaataaaagcgaaggtggacatgaaaaaaaaaaaaaaaaaaa

SEQ ID NO: 5 - protein, 801 aa, Homo sapiens; identical to SEQ ID NO: 1

SEQ ID NO: 6 - DNA, 3506 bp, Homo sapiens
  CDS (284)..(2530)
tttcaaacagcggaacaaactgaaagctccggtgccagaccccacccccggccccggcccgggaccccctcccctcccgggatcccccggggttcccaccccgcccgcaccgccggggacccggccggtccggcgcgagcccccgtccggggccctggctcggcccccaggttggaggagcccggagcccgccttcggagctacggcctaacggcggcggcgactgcagtctggagggtccacacttgtgattctcaatggagagtgaaaacgcagattcataatgaaaactagcccccgtcggccactgattctcaaaagacggaggctgccccttcctgttcaaaatgccccaagtgaaacatcagaggaggaacctaagagatcccctgcccaacaggagtctaatcaagcagaggcctccaaggaagtggcagagtccaactcttgcaagtttccagctgggatcaagattattaaccaccccaccatgcccaacacgcaagtagtggccatccccaacaatgctaatattcacagcatcatcacagcactgactgccaagggaaaagagagtggcagtagtgggcccaacaaattcatcctcatcagctgtgggggagccccaactcagcctccaggactccggcctcaaacccaaaccagctatgatgccaaaaggacagaagtgaccctggagaccttgggaccaaaacctgcagctagggatgtgaatcttcctagaccacctggagccctttgcgagcagaaacgggagacctgtgcagatggtgaggcagcaggctgcactatcaacaatagcctatccaacatccagtggcttcgaaagatgagttctgatggactgggctcccgcagcatcaagcaagagatggaggaaaaggagaattgtcacctggagcagcgacaggttaaggttgaggagccttcgagaccatcagcgtcctggcagaactctgtgtctgagcggccaccctactcttacatggccatgatacaattcgccatcaacagcactgagaggaagcgcatgactttgaaagacatctatacgtggattgaggaccactttccctactttaagcacattgccaagccaggctggaagaactccatccgccacaacctttccctgcacgacatgtttgtccgggagacgtctgccaatggcaaggtctccttctggaccattcaccccagtgccaaccgctacttgacattggaccaggtgtttaagcagcagaaacgaccgaatccagagctccgccggaacatgaccatcaaaaccgaactccccctgggcgcacggcggaagatgaagccactgctaccacgggtcagctcatacctggtacctatccagttcccggtgaaccagtcactggtgttgcagccctcggtgaaggtgccattgcccctggcggcttccctcatgagctcagagcttgcccgccatagcaagcgagtccgcattgcccccaaggtgctgctagctgaggaggggatagctcctctttcttctgcaggaccagggaaagaggagaaactcctgtttggagaagggttttctcctttgcttccagttcagactatcaaggaggaagaaatccagcctggggaggaaatgccacacttagcgagacccatcaaagtggagagccctcccttggaagagtggccctccccggccccatctttcaaagaggaatcatctcactcctgggaggattcgtcccaatctcccaccccaagacccaagaagtcctacagtgggcttaggtccccaacccggtgtgtctcggaaatgcttgtgattcaacacagggagaggagggagaggagccggtctcggaggaaacagcatctactgcctccctgtgtggatgagccggagctgctcttctcagaggggcccagtacttcccgctgggccgcagagctcccgttcccagcagactcctctgaccctgcctcccagctcagctactcccaggaagtgggaggaccttttaagacacccattaaggaaacgctgcccatctcctccaccccgagcaaatctgtcctccccagaacccctgaatcctggaggctcacgcccccagccaaagtagggggactggatttcagcccagtacaaacctcccagggtgcctctgaccccttgcctgaccccctggggctgatggatctcagcaccactcccttgcaaagtgctcccccccttgaatcaccgcaaaggctcctcagttcagaacccttagacctcatctccgtcccctttggcaactcttctccctcagatatagacgtccccaagccaggctccccggagccacaggtttctggccttgcagccaatcgttctctgacagaaggcctggtcctggacacaatgaatgacagcctcagcaagatcctgctggacatcagctttcctggcctggacgaggacccactgggccctgacaacatcaactggtcccagtttattcctgagctacagtagagccctgcccttgcccctgtgctcaagctgtccaccatcccgggcactccaaggctcagtgcaccccaagcctctgagtgaggacagcaggcagggactgttctgctcctcatagctccctgctgcctgattatgcaaaagtagcagtcacaccctagccactgctgggaccttgtgttccccaagagtatctgattcctctgctgtccctgccaggagctgaagggtgggaacaacaaaggcaatggtgaaaagagattaggaaccccccagcctgtttccattctctgcccagcagtctcttaccttccctgatctttgcagggtggtccgtgtaaatagtataaattctccaaattatcctctaattataaatgtaagcttatttccttagatcattatccagagactgccagaaggtgggtaggatgacctggggtttcaattgacttctgttccttgcttttagttttgatagaagggaagacctgcagtgcacggtttcttccaggctgaggtacctggatcttgggttcttcactgcagggacccagacaagtggatctgcttgccagagtcctttttgcccctccctgccacctccccgtgtttccaagtcagctttcctgcaagaagaaatcctggttaaaaaagtcttttgtattgggtcaggagttgaatttggggtgggaggatggatgcaactgaagcagagtgtgggtgcccagatgtgcgctattagatgtttctctgataatgtccccaatcataccagggagactggcattgacgagaactcaggtggaggcttgagaaggccgaaagggcccctgacctgcctggcttccttagcttgcccctcagctttgcaaagagccaccctaggccccagctgaccgcatgggtgtgagccagcttgagaacactaactactcaataaaagcgaaggtggacatgaaaaaaaaaaaaaaaaaaa